European Patent Application EP 4 122 491 A1, published January 25, 2023. Title: Recombinant Mycobacterium as an immunotherapeutic agent for the second-line therapy of bladder carcinoma. Applicant: Vakzine Projekt Management GmbH Serum Institute of India, Ltd. The sequence listing filed with the application follows.

SEQUENCE LISTING (2 sequences)

SEQ ID NO: 1 - DNA, 1881 bp, Artificial Sequence
  source 1..1881: /mol_type="DNA" /note="recombinant nucleic acid molecule" /organism="Artificial Sequence"
  source 1..1881: /mol_type="DNA" /note="CDS comprising a phagolysosomal domain (211-1722nt) and a stop codon (1879-1881)" /organism="Artificial Sequence"
atgacagacgtgagccgaaagattcgagcttggggacgccgattgatgatcggcacggcagcggctgtagtccttccgggcctggtggggcttgccggcggagcggcaaccgcgggcgcgttctcccggccggggctgccggtcgagtacctgcagtctgcaaagcaatccgctgcaaataaattgcactcagcaggacaaagcacgaaagatgcatctgcattcaataaagaaaattcaatttcatccatggcaccaccagcatctccgcctgcaagtcctaagacgccaatcgaaaagaaacacgcggatgaaatcgataagtatatacaaggattggattacaataaaaacaatgtattagtataccacggagatgcagtgacaaatgtgccgccaagaaaaggttacaaagatggaaatgaatatattgttgtggagaaaaagaagaaatccatcaatcaaaataatgcagacattcaagttgtgaatgcaatttcgagcctaacctatccaggtgctctcgtaaaagcgaattcggaattagtagaaaatcaaccagatgttctccctgtaaaacgtgattcattaacactcagcattgatttgccaggtatgactaatcaagacaataaaatcgttgtaaaaaatgccactaaatcaaacgttaacaacgcagtaaatacattagtggaaagatggaatgaaaaatatgctcaagcttatccaaatgtaagtgcaaaaattgattatgatgacgaaatggcttacagtgaatcacaattaattgcgaaatttggtacagcatttaaagctgtaaataatagcttgaatgtaaacttcggcgcaatcagtgaagggaaaatgcaagaagaagtcattagttttaaacaaatttactataacgtgaatgttaatgaacctacaagaccttccagatttttcggcaaagctgttactaaagagcagttgcaagcgcttggagtgaatgcagaaaatcctcctgcatatatctcaagtgtggcgtatggccgtcaagtttatttgaaattatcaactaattcccatagtactaaagtaaaagctgcttttgatgctgccgtaagcggaaaatctgtctcaggtgatgtagaactaacaaatatcatcaaaaattcttccttcaaagccgtaatttacggaggttccgcaaaagatgaagttcaaatcatcgacggcaacctcggagacttacgcgatattttgaaaaaaggcgctacttttaatcgagaaacaccaggagttcccattgcttatacaacaaacttcctaaaagacaatgaattagctgttattaaaaacaactcagaatatattgaaacaacttcaaaagcttatacagatggaaaaattaacatcgatcactctggaggatacgttgctcaattcaacatttcttgggatgaagtaaattatgatcctgaaggtaacgaaattgttcaacataaaaactggagcgaaaacaataaaagcaagctagctcatttcacatcgtccatctatttgccaggtaacgcgagaaatattaatgtttacgctaaagaatgcactggtttagcttgggaatggtggagaacggtaattgatgaccggaacttaccacttgtgaaaaatagaaatatctccatctggggcaccacgctttatccgaaatatagtaataaagtagataatccaatcgaatatgcattagcctatggaagtcagggtgatcttaatccattaattaatgaaatcagcaaaatcatttcagctgcagttctttcctctttaacatcgaagctacctgcagagttcgttaggcgcggatccggaattcgaagcttatcgatgtcgacgtag

SEQ ID NO: 2 - protein, 626 aa, Artificial Sequence
  SOURCE 1..626: /mol_type="protein" /note="CORRESPONDING AMINO ACID SEQUENCE OF SEQ ID NO: 1." /organism="Artificial Sequence"
MTDVSRKIRAWGRRLMIGTAAAVVLPGLVGLAGGAATAGAFSRPGLPVEYLQSAKQSAANKLHSAGQSTKDASAFNKENSISSMAPPASPPASPKTPIEKKHADEIDKYIQGLDYNKNNVLVYHGDAVTNVPPRKGYKDGNEYIVVEKKKKSINQNNADIQVVNAISSLTYPGALVKANSELVENQPDVLPVKRDSLTLSIDLPGMTNQDNKIVVKNATKSNVNNAVNTLVERWNEKYAQAYPNVSAKIDYDDEMAYSESQLIAKFGTAFKAVNNSLNVNFGAISEGKMQEEVISFKQIYYNVNVNEPTRPSRFFGKAVTKEQLQALGVNAENPPAYISSVAYGRQVYLKLSTNSHSTKVKAAFDAAVSGKSVSGDVELTNIIKNSSFKAVIYGGSAKDEVQIIDGNLGDLRDILKKGATFNRETPGVPIAYTTNFLKDNELAVIKNNSEYIETTSKAYTDGKINIDHSGGYVAQFNISWDEVNYDPEGNEIVQHKNWSENNKSKLAHFTSSIYLPGNARNINVYAKECTGLAWEWWRTVIDDRNLPLVKNRNISIWGTTLYPKYSNKVDNPIEYALAYGSQGDLNPLINEISKIISAAVLSSLTSKLPAEFVRRGSGIRSLSMST